European Patent Specification EP 3 959 344 B1, published June 4, 2025. Title: Systems and Methods for Targeting Dirofilaria Immitis and Dirofilaria Repens. Applicant: Smith College Saunders, Lori J. Williams, Steven A. Pilotte, Nils. The sequence listing filed with the application follows.

SEQUENCE LISTING (30 sequences)

SEQ ID NO: 1 - DNA, 71 bp, Dirofilaria immitis
acgatgaatttgtcgtatatatttgtataattcatagatacgcattgtgactcgtctaatcatatatatat

SEQ ID NO: 2 - DNA, 71 bp, Dirofilaria immitis
atatatatatgattagacgagtcacaatgcgtatctatgaattatacaaatatatacgacaaattcatcgt

SEQ ID NO: 3 - DNA, 26 bp, Artificial Sequence
  5'-biotin
acgatgaatttgtcgtatatatttgt

SEQ ID NO: 4 - DNA, 21 bp, Artificial Sequence
  5'-biotin
tgattagacgagtcacaatgc

SEQ ID NO: 5 - DNA, 211 bp, Dirofilaria repens
ttggtaataagacttaataaattttaatctcaaatatttccttgttaatatatctggtgttctattgttatatatattccggtagaccatgaaatgatgtttttattattgtacattatcaaactctggtaaaccaaatgtccaagaaccgatgcattaaatgaaaacagaaaccttggtaataagacttaataaattttaatctcaaata

SEQ ID NO: 6 - DNA, 211 bp, Dirofilaria repens
tatttgagattaaaatttattaagtcttattaccaaggtttctgttttcatttaatgcatcggttcttggacatttggtttaccagagtttgataatgtacaataataaaaacatcatttcatggtctaccggaatatatataacaatagaacaccagatatattaacaaggaaatatttgagattaaaatttattaagtcttattaccaa

SEQ ID NO: 7 - DNA, 26 bp, Artificial Sequence
  5'-biotin
tccttgttaatatatctggtgttcta

SEQ ID NO: 8 - DNA, 22 bp, Artificial Sequence
  5'-biotin
ggttcttggacatttggtttac

SEQ ID NO: 9 - DNA, 26 bp, Artificial Sequence
  Synthetic construct
acgatgaatttgtcgtatatatttgt

SEQ ID NO: 10 - DNA, 21 bp, Artificial Sequence
  Synthetic construct
tgattagacgagtcacaatgc

SEQ ID NO: 11 - DNA, 26 bp, Artificial Sequence
  5'-6-FAM fluorescent dye       3'-Iowa Black FQ quencher       Internal ZEN quencher 9 bases from the 5' end
tcatagatacgcattgtgactcgtct

SEQ ID NO: 12 - DNA, 26 bp, Artificial Sequence
  Synthetic construct
tccttgttaatatatctggtgttcta

SEQ ID NO: 13 - DNA, 22 bp, Artificial Sequence
  Synthetic construct
ggttcttggacatttggtttac

SEQ ID NO: 14 - DNA, 30 bp, Artificial Sequence
  5'-6-FAM fluorescent dye       3'-Iowa Black FQ quencher       Internal ZEN quencher 9 bases from the 5' end
tatattccggtagaccatgaaatgatgttt

SEQ ID NO: 15 - DNA, 20 bp, Artificial Sequence
  Synthetic construct
ttccggtagaccatgaaatg

SEQ ID NO: 16 - DNA, 24 bp, Artificial Sequence
  Synthetic construct
gtcttattaccaaggtttctgttt

SEQ ID NO: 17 - DNA, 30 bp, Artificial Sequence
  5'-6-FAM fluorescent dye       3'-Iowa Black FQ quencher       Internal ZEN quencher 9 bases from the 5' end
cattatcaaactctggtaaaccaaatgtcc

SEQ ID NO: 18 - DNA, 28 bp, Artificial Sequence
  Synthetic construct
ctattgttatatatattccggtagacca

SEQ ID NO: 19 - DNA, 19 bp, Artificial Sequence
  Synthetic construct
gcatcggttcttggacatt

SEQ ID NO: 20 - DNA, 29 bp, Artificial Sequence
  5'-6-FAM fluorescent dye       3'-Iowa Black FQ quencher       Internal ZEN quencher 9 bases from the 5' end
attgtacattatcaaactctggtaaacca

SEQ ID NO: 21 - DNA, 21 bp, Artificial Sequence
  Synthetic construct
cgagtcacaatgcgtatctat

SEQ ID NO: 22 - DNA, 24 bp, Artificial Sequence
  5'-6-FAM fluorescent dye       3'-Iowa Black FQ quencher       Internal ZEN quencher 9 bases from the 5' end
acgcattgtgactcgtctaatcat

SEQ ID NO: 23 - DNA, 26 bp, Artificial Sequence
  Synthetic construct
atatatatatgattagacgagtcaca

SEQ ID NO: 24 - DNA, 29 bp, Artificial Sequence
  5'-6-FAM fluorescent dye       3'-Iowa Black FQ quencher       Internal ZEN quencher 9 bases from the 5' end
aattcatagatacgcattgtgactcgtct

SEQ ID NO: 25 - DNA, 61 bp, Dirofilaria repens
atggatagaatagatatatatgtataaatataattttcaatattatttatacatgatgtat

SEQ ID NO: 26 - DNA, 131 bp, Dirofilaria repens
tagcttcgttggttttccctaagtcacgaattgctcctatcaaaggtatgactattccaagattagagttattagccgtgctcataggaatacgtggtgctcaatttgttattaaacagatgaaatagaaa

SEQ ID NO: 27 - DNA, 361 bp, Dirofilaria repens
ttaattttctctgtgccttctatgatgttattcaatgtcgtgatgatgcttctttttacagtattaagaatcttttattaattttatccgtgcattctatgatgttattcagtgtcgtgatgatgcttctttttacagtattaagaatttttctactttattgttttagaaattgtatgagttttttttgtgccttctatgatgttattcagtgtcgtgatgatgcttctttttgcagtattaagaatatttcttttattaattttctctgtgccttctatgatgttattcagtgtcgtgatgatgcttctttttacagtattaagaatttttcttttattaattttctctgtgccttcta

SEQ ID NO: 28 - DNA, 354 bp, Dirofilaria repens
tttcctatatataaaatcctatatttaaataattaattgataaaattaaatcctatatttcctatatataaaatcctatatttaaattatttgattgataaaattaaatcctatatttcctatatataaaatcctatttaaattatttgattgataaaattaaatcctatatttcctatatataaaatcctatatttaaattatttgattgataaaattaaatcctatatttcctatatataaaatcctatatttaaataattaattgataaaattaaatcctatatttcctatatataaaatcctatatttaaattatttgattgataaaattaaatcctatatttcctatat

SEQ ID NO: 29 - DNA, 26 bp, Artificial Sequence
  5'-biotin
atatatatatgattagacgagtcaca

SEQ ID NO: 30 - DNA, 23 bp, Artificial Sequence
  5' 6-FAM fluorescent dye
ttgtataattcatagatacgcat